European Patent Application EP 4 424 317 A1, published September 4, 2024. Title: 用于预防或治疗肠炎和肠癌的药物. Applicant: 安徽楚沅生物科技有限公司. The sequence listing filed with the application follows.

SEQUENCE LISTING (16 sequences)

SEQ ID NO: 1 - DNA, 22 bp, synthetic construct
  source 1..22: mol_type = other DNA
tctccagccaccagccctctaa

SEQ ID NO: 2 - DNA, 22 bp, synthetic construct
  source 1..22: mol_type = other DNA
tggccatggtaggagaaacagg

SEQ ID NO: 3 - DNA, 22 bp, synthetic construct
  source 1..22: mol_type = other DNA
acaaagccagagtccttcagag

SEQ ID NO: 4 - DNA, 17 bp, synthetic construct
  source 1..17: mol_type = other DNA
ggcagaggggttgactt

SEQ ID NO: 5 - DNA, 21 bp, synthetic construct
  source 1..21: mol_type = other DNA
tccaggatgaggacatgagca

SEQ ID NO: 6 - DNA, 21 bp, synthetic construct
  source 1..21: mol_type = other DNA
gaacgtcacacaccagcaggt

SEQ ID NO: 7 - DNA, 17 bp, synthetic construct
  source 1..17: mol_type = other DNA
aacaacgccctaaagca

SEQ ID NO: 8 - DNA, 17 bp, synthetic construct
  source 1..17: mol_type = other DNA
tggattcacataggagc

SEQ ID NO: 9 - DNA, 18 bp, synthetic construct
  source 1..18: mol_type = other DNA
cacgtatacccgctacct

SEQ ID NO: 10 - DNA, 17 bp, synthetic construct
  source 1..17: mol_type = other DNA
ccagtttcattcgagca

SEQ ID NO: 11 - DNA, 22 bp, synthetic construct
  source 1..22: mol_type = other DNA
ggcggatatacagacccaagag

SEQ ID NO: 12 - DNA, 24 bp, synthetic construct
  source 1..24: mol_type = other DNA
gataatcatgaaccccaggacaat

SEQ ID NO: 13 - DNA, 21 bp, synthetic construct
  source 1..21: mol_type = other DNA
gagcgggctaccttactgaac

SEQ ID NO: 14 - DNA, 23 bp, synthetic construct
  source 1..23: mol_type = other DNA
gtcatctctttccgaggcattag

SEQ ID NO: 15 - DNA, 20 bp, synthetic construct
  source 1..20: mol_type = other DNA
ccagtatgactccactcacg

SEQ ID NO: 16 - DNA, 20 bp, synthetic construct
  source 1..20: mol_type = other DNA
gactccacgacatactcagc